European Patent Application EP 4 470 564 A1, published December 4, 2024. Title: DRUG AND METHOD FOR NUCLEOSIDE (ACID) DRUG THERAPY OF LIMITING CHRONIC HEPATITIS B. Applicant: SHANGHAI HEP PHARMACEUTICAL CO.,LTD. The sequence listing filed with the application follows.

SEQUENCE LISTING (44 sequences)

SEQ ID NO: 1 - protein, 119 aa, synthetic construct
  REGION 1..119: note = Gene bank ID AF461363
MGGWSSKPRQGMGTNLSVPNPLGFFPDHQLDPAFGANSNNPDWDFNPNKDHWPEANQVGAGAFGPGFTPPHGGLLGWSPQAQGILTTVPVAPPPASTNRQSGRQPTPISPPLRDSHPQA

SEQ ID NO: 2 - protein, 118 aa, synthetic construct
  REGION 1..118: note = C Pre-S1(2-119)
GGWSSKPRQGMGTNLSVPNPLGFFPDHQLDPAFGANSNNPDWDFNPNKDHWPEANQVGAGAFGPGFTPPHGGLLGWSPQAQGILTTVPVAPPPASTNRQSGRQPTPISPPLRDSHPQA

SEQ ID NO: 3 - protein, 68 aa, synthetic construct
  REGION 1..68: note = C Pre-S1(2-69)
GGWSSKPRQGMGTNLSVPNPLGFFPDHQLDPAFGANSNNPDWDFNPNKDHWPEANQVGAGAFGPGFTP

SEQ ID NO: 4 - protein, 58 aa, synthetic construct
  REGION 1..58: note = C Pre-S1(2-59)
GGWSSKPRQGMGTNLSVPNPLGFFPDHQLDPAFGANSNNPDWDFNPNKDHWPEANQVG

SEQ ID NO: 5 - protein, 107 aa, synthetic construct
  REGION 1..107: note = C Pre-S1(13-119)
GTNLSVPNPLGFFPDHQLDPAFGANSNNPDWDFNPNKDHWPEANQVGAGAFGPGFTPPHGGLLGWSPQAQGILTTVPVAPPPASTNRQSGRQPTPISPPLRDSHPQA

SEQ ID NO: 6 - protein, 76 aa, synthetic construct
  REGION 1..76: note = C Pre-S1(13-88)
GTNLSVPNPLGFFPDHQLDPAFGANSNNPDWDFNPNKDHWPEANQVGAGAFGPGFTPPHGGLLGWSPQAQGILTTV

SEQ ID NO: 7 - protein, 60 aa, synthetic construct
  REGION 1..60: note = C Pre-S1(13-72)
GTNLSVPNPLGFFPDHQLDPAFGANSNNPDWDFNPNKDHWPEANQVGAGAFGPGFTPPHG

SEQ ID NO: 8 - protein, 55 aa, synthetic construct
  REGION 1..55: note = C Pre-S1(13-67)
GTNLSVPNPLGFFPDHQLDPAFGANSNNPDWDFNPNKDHWPEANQVGAGAFGPGF

SEQ ID NO: 9 - protein, 47 aa, synthetic construct
  REGION 1..47: note = C Pre-S1(13-59)
GTNLSVPNPLGFFPDHQLDPAFGANSNNPDWDFNPNKDHWPEANQVG

SEQ ID NO: 10 - protein, 40 aa, synthetic construct
  REGION 1..40: note = C Pre-S1(13-52)
GTNLSVPNPLGFFPDHQLDPAFGANSNNPDWDFNPNKDHW

SEQ ID NO: 11 - protein, 35 aa, synthetic construct
  REGION 1..35: note = C Pre-S1(13-47)
GTNLSVPNPLGFFPDHQLDPAFGANSNNPDWDFNP

SEQ ID NO: 12 - protein, 30 aa, synthetic construct
  REGION 1..30: note = C Pre-S1(13-42)
GTNLSVPNPLGFFPDHQLDPAFGANSNNPD

SEQ ID NO: 13 - protein, 25 aa, synthetic construct
  REGION 1..25: note = C Pre-S1(13-37)
GTNLSVPNPLGFFPDHQLDPAFGAN

SEQ ID NO: 14 - protein, 20 aa, synthetic construct
  REGION 1..20: note = C Pre-S1(13-32)
GTNLSVPNPLGFFPDHQLDP

SEQ ID NO: 15 - protein, 47 aa, synthetic construct
  REGION 1..47: note = C Pre-S1(13-59)
GTDLSVPNPLGFFPDHQLDPAFGANSNNPDWDFNPNKDHWPEANQVG

SEQ ID NO: 16 - protein, 47 aa, synthetic construct
  REGION 1..47: note = C Pre-S1(13-59)
GTNLSVPNPLGFLPDHQLDPAFGANSNNPDWDFNPNKDHWPEANQVG

SEQ ID NO: 17 - protein, 47 aa, synthetic construct
  REGION 1..47: note = C Pre-S1(13-59)
GTNLSVPNPLGFFPDHQLDPAFKANSNNPDWDFNPNKDHWPEANQVG

SEQ ID NO: 18 - protein, 47 aa, synthetic construct
  REGION 1..47: note = C Pre-S1(13-59)
GTNLSVPNPLGFFPDHQLDPAFGANSENPDWDFNPNKDHWPEANQVG

SEQ ID NO: 19 - protein, 47 aa, synthetic construct
  REGION 1..47: note = C Pre-S1(13-59)
GTNLSVPNPLGFFPDHQLDPAFGANSNNPDWDFKPNKDHWPEANQVG

SEQ ID NO: 20 - protein, 47 aa, synthetic construct
  REGION 1..47: note = C Pre-S1(13-59)
GTNLSVPNPLGFFPDHQLDPAFGANSNNPDWDLNPNKDHWPEANQVG

SEQ ID NO: 21 - protein, 47 aa, synthetic construct
  REGION 1..47: note = C Pre-S1(13-59)
GTNLSVPNPLGFFPDHQLDPAFGANSNNPDWDFNPHKDHWPEANQVG

SEQ ID NO: 22 - protein, 47 aa, synthetic construct
  REGION 1..47: note = C Pre-S1(13-59)
GTNLSVPNPLGFFPDHQLDPAFGANSNNPDWDFNPYKDHWPEANQVG

SEQ ID NO: 23 - protein, 47 aa, synthetic construct
  REGION 1..47: note = C Pre-S1(13-59)
GTNLSVPNPLGFFPDHQLDPAFGANSNNPDWDFNPKKDHWPEANQVG

SEQ ID NO: 24 - protein, 47 aa, synthetic construct
  REGION 1..47: note = C Pre-S1(13-59)
GTNLSVPNPLGFFPDHQLDPAFGANSNNPDWDFNPNKAHWPEANQVG

SEQ ID NO: 25 - protein, 47 aa, synthetic construct
  REGION 1..47: note = C Pre-S1(13-59)
GTNLSVPNPLGFFPDHQLDPAFGANSNNPDWDFNPNKDQWPEANQVG

SEQ ID NO: 26 - protein, 47 aa, synthetic construct
  REGION 1..47: note = C Pre-S1(13-59)
GTNLSVPNPLGFFPDHQLDPAFGANSNNPDWDFNPNKDNWPEANQVG

SEQ ID NO: 27 - protein, 47 aa, synthetic construct
  REGION 1..47: note = C Pre-S1(13-59)
GTNLSVPNPLGFFPDHQLDPAFGANSNNPDWDFNPNKDHWPKANQVG

SEQ ID NO: 28 - protein, 47 aa, synthetic construct
  REGION 1..47: note = C Pre-S1(13-59)
GTNLSVPNPLGFFPDHQLDPAFGANSNNPDWDFNPNKDHWPDANQVG

SEQ ID NO: 29 - protein, 47 aa, synthetic construct
  REGION 1..47: note = C Pre-S1(13-59)
GTNLSVPNPLGFFPDHQLDPAFGANSNNPDWDFNPNKDHWPESNQVG

SEQ ID NO: 30 - protein, 47 aa, synthetic construct
  REGION 1..47: note = C Pre-S1(13-59)
GTNLSVPNPLGFFPDHQLDPAFGANSNNPDWDFNPNKDHWPEAKQVG

SEQ ID NO: 31 - protein, 47 aa, synthetic construct
  REGION 1..47: note = C Pre-S1(13-59)
GTNLSVPNPLGFFPDHQLDPAFGANSNNPDWDFNPNKDHWPEADQVG

SEQ ID NO: 32 - protein, 47 aa, synthetic construct
  REGION 1..47: note = C Pre-S1(13-59)
GTNLSVPNPLGFFPDHQLDPAFGANSNNPDWDFNPNKDHWPEANKVG

SEQ ID NO: 33 - protein, 47 aa, synthetic construct; identical to SEQ ID NO: 9
  REGION 1..47: note = C Pre-S1(13-59)
  REGION 1..47: note = N-term Myr
  REGION 1..47: note = C-term NH2

SEQ ID NO: 34 - protein, 47 aa, synthetic construct; identical to SEQ ID NO: 32
  REGION 1..47: note = C Pre-S1(13-59)
  REGION 1..47: note = N-term Myr
  REGION 1..47: note = C-term NH2

SEQ ID NO: 35 - protein, 47 aa, synthetic construct; identical to SEQ ID NO: 9
  REGION 1..47: note = C Pre-S1(13-59)
  REGION 1..47: note = N-term Plam
  REGION 1..47: note = C-term NH2

SEQ ID NO: 36 - protein, 47 aa, synthetic construct; identical to SEQ ID NO: 9
  REGION 1..47: note = C Pre-S1(13-59)
  REGION 1..47: note = N-term Stearoyl
  REGION 1..47: note = C-term NH2

SEQ ID NO: 37 - protein, 47 aa, synthetic construct; identical to SEQ ID NO: 9
  REGION 1..47: note = C Pre-S1(13-59)
  REGION 1..47: note = N-term Chol
  REGION 1..47: note = C-term NH2

SEQ ID NO: 38 - protein, 47 aa, synthetic construct
  REGION 1..47: note = A Pre-S1(13-59)
  REGION 1..47: note = N-term Myr
  REGION 1..47: note = C-term NH2
GTNLSVPNPLGFFPDHQLDPAFGANSNNPDWDFNPVKDDWPAANQVG

SEQ ID NO: 39 - protein, 47 aa, synthetic construct
  REGION 1..47: note = B Pre-S1(13-59)
  REGION 1..47: note = N-term Myr
  REGION 1..47: note = C-term NH2
GTNLSVPNPLGFFPDHQLDPAFKANSENPDWDLNPNKDNWPDANKVG

SEQ ID NO: 40 - protein, 47 aa, synthetic construct
  REGION 1..47: note = D Pre-S1(2-48)
  REGION 1..47: note = N-term Myr
  REGION 1..47: note = C-term NH2
GQNLSTSNPLGFFPDHQLDPAFRANTANPDWDFNPNKDTWPDANKVG

SEQ ID NO: 41 - protein, 47 aa, synthetic construct
  REGION 1..47: note = E Pre-S1(12-58)
  REGION 1..47: note = N-term Myr
  REGION 1..47: note = C-term NH2
GKNISTTNPLGFFPDHQLDPAFRANTRNPDWDHNPNKDHWTEANKVG

SEQ ID NO: 42 - protein, 47 aa, synthetic construct
  REGION 1..47: note = F Pre-S1(13-59)
  REGION 1..47: note = N-term Myr
  REGION 1..47: note = C-term NH2
GQNLSVPNPLGFFPDHQLDPLFRANSSSPDWDFNTNKDSWPMANKVG

SEQ ID NO: 43 - protein, 47 aa, synthetic construct
  REGION 1..47: note = G Pre-S1(12-58)
  REGION 1..47: note = N-term Myr
  REGION 1..47: note = C-term NH2
GKNLSASNPLGFLPDHQLDPAFRANTNNPDWDFNPKKDPWPEANKVG

SEQ ID NO: 44 - protein, 47 aa, synthetic construct
  REGION 1..47: note = H Pre-S1(13-59)
  REGION 1..47: note = N-term Myr
  REGION 1..47: note = C-term NH2
GQNLSVPNPLGFFPDHQLDPLFRANSSSPDWDFNTNKDNWPMANKVG